European Patent Application EP 4 685 158 A1, published January 28, 2026. Title: Fibrillary Apolipoprotein E (ApoE) for use in a method of treatment and/or prevention of a neurodegenerative disease. Applicant: Technische Universitaet Muenchen. Application EP. The sequence listing filed with the application follows.

SEQUENCE LISTING (42 sequences)

SEQ ID NO: 1 - protein, 299 aa, synthetic construct
KVEQAVETEPEPELRQQTEWQSGQRWELALGRFWDYLRWVQTLSEQVQEELLSSQVTQELRALMDETMKELKAYKSELEEQLTPVAEETRARLSKELQAAQARLGADMEDVRGRLVQYRGEVQAMLGQSTEELRVRLASHLRKLRKRLLRDADDLQKRLAVYQAGAREGAERGLSAIRERLGPLVEQGRVRAATVGSLAGQPLQERAQAWGERLRARMEEMGSRTRDRLDEVKEQVAEVRAKLEEQAQQIRLQAEAFQARLKSWFEPLVEDMQRQWAGLVEKVQAAVGTSAAPVPSDNH

SEQ ID NO: 2 - protein, 306 aa, synthetic construct
MHHHHHHKVEQAVETEPEPELRQQTEWQSGQRWELALGRFWDYLRWVQTLSEQVQEELLSSQVTQELRALMDETMKELKAYKSELEEQLTPVAEETRARLSKELQAAQARLGADMEDVRGRLVQYRGEVQAMLGQSTEELRVRLASHLRKLRKRLLRDADDLQKRLAVYQAGAREGAERGLSAIRERLGPLVEQGRVRAATVGSLAGQPLQERAQAWGERLRARMEEMGSRTRDRLDEVKEQVAEVRAKLEEQAQQIRLQAEAFQARLKSWFEPLVEDMQRQWAGLVEKVQAAVGTSAAPVPSDNH

SEQ ID NO: 3 - protein, 305 aa, synthetic construct
HHHHHHKVEQAVETEPEPELRQQTEWQSGQRWELALGRFWDYLRWVQTLSEQVQEELLSSQVTQELRALMDETMKELKAYKSELEEQLTPVAEETRARLSKELQAAQARLGADMEDVRGRLVQYRGEVQAMLGQSTEELRVRLASHLRKLRKRLLRDADDLQKRLAVYQAGAREGAERGLSAIRERLGPLVEQGRVRAATVGSLAGQPLQERAQAWGERLRARMEEMGSRTRDRLDEVKEQVAEVRAKLEEQAQQIRLQAEAFQARLKSWFEPLVEDMQRQWAGLVEKVQAAVGTSAAPVPSDNH

SEQ ID NO: 4 - protein, 612 aa, synthetic construct
MKVEQAVETEPEPELRQQTEWQSGQRWELALGRFWDYLRWVQTLSEQVQEELLSSQVTQELRALMDETMKELKAYKSELEEQLTPVAEETRARLSKELQAAQARLGADMEDVRGRLVQYRGEVQAMLGQSTEELRVRLASHLRKLRKRLLRDADDLQKRLAVYQAGAREGAERGLSAIRERLGPLVEQGRVRAATVGSLAGQPLQERAQAWGERLRARMEEMGSRTRDRLDEVKEQVAEVRAKLEEQAQQIRLQAEAFQARLKSWFEPLVEDMQRQWAGLVEKVQAAVGTSAAPVPSDNHLEPTTEDLYFQSDNDGSEIGTGFPFDPHYVEVLGERMHYVDVGPRDGTPVLFLHGNPTSSYVWRNIIPHVAPTHRCIAPDLIGMGKSDKPDLGYFFDDHVRFMDAFIEALGLEEVVLVIHDWGSALGFHWAKRNPERVKGIAFMEFIRPIPTWDEWPEFARETFQAFRTTDVGRKLIIDQNVFIEGTLPMGVVRPLTEVEMDHYREPFLNPVDREPLWRFPNELPIAGEPANIVALVEEYMDWLHQSPVPKLLFWGTPGVLIPPAEAARLAKSLPNCKAVDIGPGLNLLQEDNPDLIGSEIARWLSTLEISG

SEQ ID NO: 5 - protein, 611 aa, synthetic construct
KVEQAVETEPEPELRQQTEWQSGQRWELALGRFWDYLRWVQTLSEQVQEELLSSQVTQELRALMDETMKELKAYKSELEEQLTPVAEETRARLSKELQAAQARLGADMEDVRGRLVQYRGEVQAMLGQSTEELRVRLASHLRKLRKRLLRDADDLQKRLAVYQAGAREGAERGLSAIRERLGPLVEQGRVRAATVGSLAGQPLQERAQAWGERLRARMEEMGSRTRDRLDEVKEQVAEVRAKLEEQAQQIRLQAEAFQARLKSWFEPLVEDMQRQWAGLVEKVQAAVGTSAAPVPSDNHLEPTTEDLYFQSDNDGSEIGTGFPFDPHYVEVLGERMHYVDVGPRDGTPVLFLHGNPTSSYVWRNIIPHVAPTHRCIAPDLIGMGKSDKPDLGYFFDDHVRFMDAFIEALGLEEVVLVIHDWGSALGFHWAKRNPERVKGIAFMEFIRPIPTWDEWPEFARETFQAFRTTDVGRKLIIDQNVFIEGTLPMGVVRPLTEVEMDHYREPFLNPVDREPLWRFPNELPIAGEPANIVALVEEYMDWLHQSPVPKLLFWGTPGVLIPPAEAARLAKSLPNCKAVDIGPGLNLLQEDNPDLIGSEIARWLSTLEISG

SEQ ID NO: 6 - protein, 299 aa, synthetic construct
KVEQAVETEPEPELRQQTEWQSGQRWELALGRFWDYLRWVQTLSEQVQEELLSSQVTQELRALMDETMKELKAYKSELEEQLTPVAEETRARLSKELQAAQARLGADMEDVCGRLVQYRGEVQAMLGQSTEELRVRLASHLRKLRKRLLRDADDLQKCLAVYQAGAREGAERGLSAIRERLGPLVEQGRVRAATVGSLAGQPLQERAQAWGERLRARMEEMGSRTRDRLDEVKEQVAEVRAKLEEQAQQIRLQAEAFQARLKSWFEPLVEDMQRQWAGLVEKVQAAVGTSAAPVPSDNH

SEQ ID NO: 7 - protein, 306 aa, synthetic construct
MHHHHHHKVEQAVETEPEPELRQQTEWQSGQRWELALGRFWDYLRWVQTLSEQVQEELLSSQVTQELRALMDETMKELKAYKSELEEQLTPVAEETRARLSKELQAAQARLGADMEDVCGRLVQYRGEVQAMLGQSTEELRVRLASHLRKLRKRLLRDADDLQKCLAVYQAGAREGAERGLSAIRERLGPLVEQGRVRAATVGSLAGQPLQERAQAWGERLRARMEEMGSRTRDRLDEVKEQVAEVRAKLEEQAQQIRLQAEAFQARLKSWFEPLVEDMQRQWAGLVEKVQAAVGTSAAPVPSDNH

SEQ ID NO: 8 - protein, 305 aa, synthetic construct
HHHHHHKVEQAVETEPEPELRQQTEWQSGQRWELALGRFWDYLRWVQTLSEQVQEELLSSQVTQELRALMDETMKELKAYKSELEEQLTPVAEETRARLSKELQAAQARLGADMEDVCGRLVQYRGEVQAMLGQSTEELRVRLASHLRKLRKRLLRDADDLQKCLAVYQAGAREGAERGLSAIRERLGPLVEQGRVRAATVGSLAGQPLQERAQAWGERLRARMEEMGSRTRDRLDEVKEQVAEVRAKLEEQAQQIRLQAEAFQARLKSWFEPLVEDMQRQWAGLVEKVQAAVGTSAAPVPSDNH

SEQ ID NO: 9 - protein, 612 aa, synthetic construct
MKVEQAVETEPEPELRQQTEWQSGQRWELALGRFWDYLRWVQTLSEQVQEELLSSQVTQELRALMDETMKELKAYKSELEEQLTPVAEETRARLSKELQAAQARLGADMEDVCGRLVQYRGEVQAMLGQSTEELRVRLASHLRKLRKRLLRDADDLQKCLAVYQAGAREGAERGLSAIRERLGPLVEQGRVRAATVGSLAGQPLQERAQAWGERLRARMEEMGSRTRDRLDEVKEQVAEVRAKLEEQAQQIRLQAEAFQARLKSWFEPLVEDMQRQWAGLVEKVQAAVGTSAAPVPSDNHLEPTTEDLYFQSDNDGSEIGTGFPFDPHYVEVLGERMHYVDVGPRDGTPVLFLHGNPTSSYVWRNIIPHVAPTHRCIAPDLIGMGKSDKPDLGYFFDDHVRFMDAFIEALGLEEVVLVIHDWGSALGFHWAKRNPERVKGIAFMEFIRPIPTWDEWPEFARETFQAFRTTDVGRKLIIDQNVFIEGTLPMGVVRPLTEVEMDHYREPFLNPVDREPLWRFPNELPIAGEPANIVALVEEYMDWLHQSPVPKLLFWGTPGVLIPPAEAARLAKSLPNCKAVDIGPGLNLLQEDNPDLIGSEIARWLSTLEISG

SEQ ID NO: 10 - protein, 611 aa, synthetic construct
KVEQAVETEPEPELRQQTEWQSGQRWELALGRFWDYLRWVQTLSEQVQEELLSSQVTQELRALMDETMKELKAYKSELEEQLTPVAEETRARLSKELQAAQARLGADMEDVCGRLVQYRGEVQAMLGQSTEELRVRLASHLRKLRKRLLRDADDLQKCLAVYQAGAREGAERGLSAIRERLGPLVEQGRVRAATVGSLAGQPLQERAQAWGERLRARMEEMGSRTRDRLDEVKEQVAEVRAKLEEQAQQIRLQAEAFQARLKSWFEPLVEDMQRQWAGLVEKVQAAVGTSAAPVPSDNHLEPTTEDLYFQSDNDGSEIGTGFPFDPHYVEVLGERMHYVDVGPRDGTPVLFLHGNPTSSYVWRNIIPHVAPTHRCIAPDLIGMGKSDKPDLGYFFDDHVRFMDAFIEALGLEEVVLVIHDWGSALGFHWAKRNPERVKGIAFMEFIRPIPTWDEWPEFARETFQAFRTTDVGRKLIIDQNVFIEGTLPMGVVRPLTEVEMDHYREPFLNPVDREPLWRFPNELPIAGEPANIVALVEEYMDWLHQSPVPKLLFWGTPGVLIPPAEAARLAKSLPNCKAVDIGPGLNLLQEDNPDLIGSEIARWLSTLEISG

SEQ ID NO: 11 - protein, 299 aa, synthetic construct
KVEQAVETEPEPELRQQTEWQSGQRWELALGRFWDYLRWVQTLSEQVQEELLSSQVTQELRALMDETMKELKAYKSELEEQLTPVAEETRARLSKELQAAQARLGADMEDVCGRLVQYRGEVQAMLGQSTEELRVRLASHLRKLRKRLLRDADDLQKRLAVYQAGAREGAERGLSAIRERLGPLVEQGRVRAATVGSLAGQPLQERAQAWGERLRARMEEMGSRTRDRLDEVKEQVAEVRAKLEEQAQQIRLQAEAFQARLKSWFEPLVEDMQRQWAGLVEKVQAAVGTSAAPVPSDNH

SEQ ID NO: 12 - protein, 306 aa, synthetic construct
MHHHHHHKVEQAVETEPEPELRQQTEWQSGQRWELALGRFWDYLRWVQTLSEQVQEELLSSQVTQELRALMDETMKELKAYKSELEEQLTPVAEETRARLSKELQAAQARLGADMEDVCGRLVQYRGEVQAMLGQSTEELRVRLASHLRKLRKRLLRDADDLQKRLAVYQAGAREGAERGLSAIRERLGPLVEQGRVRAATVGSLAGQPLQERAQAWGERLRARMEEMGSRTRDRLDEVKEQVAEVRAKLEEQAQQIRLQAEAFQARLKSWFEPLVEDMQRQWAGLVEKVQAAVGTSAAPVPSDNH

SEQ ID NO: 13 - protein, 305 aa, synthetic construct
HHHHHHKVEQAVETEPEPELRQQTEWQSGQRWELALGRFWDYLRWVQTLSEQVQEELLSSQVTQELRALMDETMKELKAYKSELEEQLTPVAEETRARLSKELQAAQARLGADMEDVCGRLVQYRGEVQAMLGQSTEELRVRLASHLRKLRKRLLRDADDLQKRLAVYQAGAREGAERGLSAIRERLGPLVEQGRVRAATVGSLAGQPLQERAQAWGERLRARMEEMGSRTRDRLDEVKEQVAEVRAKLEEQAQQIRLQAEAFQARLKSWFEPLVEDMQRQWAGLVEKVQAAVGTSAAPVPSDNH

SEQ ID NO: 14 - protein, 612 aa, synthetic construct
MKVEQAVETEPEPELRQQTEWQSGQRWELALGRFWDYLRWVQTLSEQVQEELLSSQVTQELRALMDETMKELKAYKSELEEQLTPVAEETRARLSKELQAAQARLGADMEDVCGRLVQYRGEVQAMLGQSTEELRVRLASHLRKLRKRLLRDADDLQKRLAVYQAGAREGAERGLSAIRERLGPLVEQGRVRAATVGSLAGQPLQERAQAWGERLRARMEEMGSRTRDRLDEVKEQVAEVRAKLEEQAQQIRLQAEAFQARLKSWFEPLVEDMQRQWAGLVEKVQAAVGTSAAPVPSDNHLEPTTEDLYFQSDNDGSEIGTGFPFDPHYVEVLGERMHYVDVGPRDGTPVLFLHGNPTSSYVWRNIIPHVAPTHRCIAPDLIGMGKSDKPDLGYFFDDHVRFMDAFIEALGLEEVVLVIHDWGSALGFHWAKRNPERVKGIAFMEFIRPIPTWDEWPEFARETFQAFRTTDVGRKLIIDQNVFIEGTLPMGVVRPLTEVEMDHYREPFLNPVDREPLWRFPNELPIAGEPANIVALVEEYMDWLHQSPVPKLLFWGTPGVLIPPAEAARLAKSLPNCKAVDIGPGLNLLQEDNPDLIGSEIARWLSTLEISG

SEQ ID NO: 15 - protein, 611 aa, synthetic construct
KVEQAVETEPEPELRQQTEWQSGQRWELALGRFWDYLRWVQTLSEQVQEELLSSQVTQELRALMDETMKELKAYKSELEEQLTPVAEETRARLSKELQAAQARLGADMEDVCGRLVQYRGEVQAMLGQSTEELRVRLASHLRKLRKRLLRDADDLQKRLAVYQAGAREGAERGLSAIRERLGPLVEQGRVRAATVGSLAGQPLQERAQAWGERLRARMEEMGSRTRDRLDEVKEQVAEVRAKLEEQAQQIRLQAEAFQARLKSWFEPLVEDMQRQWAGLVEKVQAAVGTSAAPVPSDNHLEPTTEDLYFQSDNDGSEIGTGFPFDPHYVEVLGERMHYVDVGPRDGTPVLFLHGNPTSSYVWRNIIPHVAPTHRCIAPDLIGMGKSDKPDLGYFFDDHVRFMDAFIEALGLEEVVLVIHDWGSALGFHWAKRNPERVKGIAFMEFIRPIPTWDEWPEFARETFQAFRTTDVGRKLIIDQNVFIEGTLPMGVVRPLTEVEMDHYREPFLNPVDREPLWRFPNELPIAGEPANIVALVEEYMDWLHQSPVPKLLFWGTPGVLIPPAEAARLAKSLPNCKAVDIGPGLNLLQEDNPDLIGSEIARWLSTLEISG

SEQ ID NO: 16 - protein, 6 aa, synthetic construct
HHHHHH

SEQ ID NO: 17 - protein, 295 aa, synthetic construct
EIGTGFPFDPHYVEVLGERMHYVDVGPRDGTPVLFLHGNPTSSYVWRNIIPHVAPTHRCIAPDLIGMGKSDKPDLGYFFDDHVRFMDAFIEALGLEEVVLVIHDWGSALGFHWAKRNPERVKGIAFMEFIRPIPTWDEWPEFARETFQAFRTTDVGRKLIIDQNVFIEGTLPMGVVRPLTEVEMDHYREPFLNPVDREPLWRFPNELPIAGEPANIVALVEEYMDWLHQSPVPKLLFWGTPGVLIPPAEAARLAKSLPNCKAVDIGPGLNLLQEDNPDLIGSEIARWLSTLEISG

SEQ ID NO: 18 - protein, 8 aa, synthetic construct
DYKDDDDK

SEQ ID NO: 19 - protein, 22 aa, synthetic construct
DYKDHDGDYKDHDIDYKDDDDK

SEQ ID NO: 20 - protein, 9 aa, synthetic construct
YPYDVPDYA

SEQ ID NO: 21 - protein, 30 aa, synthetic construct
YPYDVPDYAGYPYDVPDYAGSYPYDVPDYA

SEQ ID NO: 22 - protein, 10 aa, synthetic construct
EQKLISEEDL

SEQ ID NO: 23 - protein, 9 aa, synthetic construct
IPNPLLGLD

SEQ ID NO: 24 - protein, 14 aa, synthetic construct
GKPIPNPLLGLDST

SEQ ID NO: 25 - protein, 15 aa, synthetic construct
GGGGSGGGGSGGGGS

SEQ ID NO: 26 - protein, 5 aa, synthetic construct
GGGGS

SEQ ID NO: 27 - protein, 8 aa, synthetic construct
GGGGGGGG

SEQ ID NO: 28 - protein, 10 aa, synthetic construct
EAAAKEAAAK

SEQ ID NO: 29 - protein, 5 aa, synthetic construct
PAPAP

SEQ ID NO: 30 - protein, 4 aa, synthetic construct
  MOTIF 1..2: note = The Ala-Pro(1) linker consists of the first two amino acids: AP. The second "AP" also displayed in the sequence, is not a mandatory feature of the AP-Linker.
APAP

SEQ ID NO: 31 - protein, 17 aa, synthetic construct
LEPTTEDLYFQSDNDGS

SEQ ID NO: 32 - protein, 7 aa, synthetic construct
ENLYFQG

SEQ ID NO: 33 - protein, 12 aa, synthetic construct
CRRRRRREAEAC

SEQ ID NO: 34 - protein, 20 aa, synthetic construct
LEAGCKNFFPRSFTSCGSLE

SEQ ID NO: 35 - protein, 8 aa, synthetic construct
WSHPQFEK

SEQ ID NO: 36 - protein, 9 aa, synthetic construct
RRRRRRRRR

SEQ ID NO: 37 - protein, 9 aa, synthetic construct
AWRHPQFGG

SEQ ID NO: 38 - protein, 36 aa, synthetic construct
QQTVWGQCGGQGWSGPTSCVAGSACSTLNPYYAQCI

SEQ ID NO: 39 - protein, 12 aa, synthetic construct
PDRVRAVSHWSS

SEQ ID NO: 40 - protein, 4 aa, synthetic construct
EPEA

SEQ ID NO: 41 - protein, 13 aa, synthetic construct
SRLEEELRRRLTE

SEQ ID NO: 42 - protein, 15 aa, synthetic construct
GLNDIFEAQKIEWHE